European Patent Specification EP 3 362 577 B1, published July 3, 2024. Title: METHODS AND KITS FOR HIGHLY MULTIPLEX SINGLE PRIMER EXTENSION. Applicant: Qiagen Sciences LLC Wang, Yexun Peng, Quan. Application PCT. The sequence listing filed with the application follows.

SEQUENCE LISTING (6 sequences)

SEQ ID NO: 1 - protein, 853 aa, Escherichia coli
MSAIENFDAHTPMMQQYLRLKAQHPEILLFYRMGDFYELFYDDAKRASQLLDISLTKRGASAGEPIPMAGIPYHAVENYLAKLVNQGESVAICEQIGDPATSKGPVERKVVRIVTPGTISDEALLQERQDNLLAAIWQDSKGFGYATLDISSGRFRLSEPADRETMAAELQRTNPAELLYAEDFAEMSLIEGRRGLRRRPLWEFEIDTARQQLNLQFGTRDLVGFGVENAPRGLCAAGCLLQYAKDTQRTTLPHIRSITMEREQDSIIMDAATRRNLEITQNLAGGAENTLASVLDCTVTPMGSRMLKRWLHMPVRDTRVLLERQQTIGALQDFTAGLQPVLRQVGDLERILARLALRTARPRDLARMRHAFQQLPELRAQLETVDSAPVQALREKMGEFAELRDLLERAIIDTPPVLVRDGGVIASGYNEELDEWRALADGATDYLERLEVRERERTGLDTLKVGFNAVHGYYIQISRGQSHLAPINYMRRQTLKNAERYIIPELKEYEDKVLTSKGKALALEKQLYEELFDLLLPHLEALQQSASALAELDVLVNLAERAYTLNYTCPTFIDKPGIRITEGRHPVVEQVLNEPFIANPLNLSPQRRMLIITGPNMGGKSTYMRQTALIALMAYIGSYVPAQKVEIGPIDRIFTRVGAADDLASGRSTFMVEMTETANILHNATEYSLVLMDEIGRGTSTYDGLSLAWACAENLANKIKALTLFATHYFELTQLPEKMEGVANVHLDALEHGDTIAFMHSVQDGAASKSYGLAVAALAGVPKEVIKRARQKLRELESISPNAAATQVDGTQMSLLSVPEETSPAVEALENLDPDSLTPRQALEWIYRLKSLV

SEQ ID NO: 2 - protein, 811 aa, Thermus aquaticus
MEGMLKGEGPGPLPPLLQQYVELRDQYPDYLLLFQVGDFYECFGEDAERLARALGLVLTHKTSKDFTTPMAGIPLRAFEAYAERLLKMGFRLAVADQVEPAEEAEGLVRREVTQLLTPGTLLQESLLPREANYLAAIATGDGWGLAFLDVSTGEFKGTVLKSKSALYDELFRHRPAEVLLAPELLENGAFLDEFRKRFPVMLSEAPFEPEGEGPLALRRARGALLAYAQRTQGGALSLQPFRFYDPGAFMRLPEATLRALEVFEPLRGQDTLFSVLDETRTAPGRRLLQSWLRHPLLDRGPLEARLDRVEGFVREGALREGVRRLLYRLADLERLATRLELGRASPKDLGALRRSLQILPELRALLGEEVGLPDLSPLKEELEAALVEDPPLKVSEGGLIREGYDPDLDALRAAHREGVAYFLELEERERERTGIPTLKVGYNAVFGYYLEVTRPYYERVPKEYRPVQTLKDRQRYTLPEMKEKEREVYRLEALIRRREEEVFLEVRERAKRQAEALREAARILAELDVYAALAEVAVRYGYVRPRFGDRLQIRAGRHPVVERRTEFVPNDLEMAHELVLITGPNMAGKSTFLRQTALIALLAQVGSFVPAEEAHLPLFDGIYTRIGASDDLAGGKSTFMVEMEEVALILKEATENSLVLLDEVGRGTSSLDGVAIATAVAEALHERRAYTLFATHYFELTALGLPRLKNLHVAAREEAGGLVFYHQVLPGPASKSYGVEVAAMAGLPKEVVARARALLQAMAARREGALDAVLERLLALDPDRLTPLEALRLLQELKALALGAPLDTMKG

SEQ ID NO: 3 - protein, 819 aa, Thermus thermophilus
MGGYGGVKMEGMLKGEGPGPLPPLLQQYVELRDRYPDYLLLFQVGDFYECFGEDAERLARALGLVLTHKTSKDFTTPMAGIPIRAFDAYAERLLKMGFRLAVADQVEPAEEAEGLVRREVTQLLTPGTLTQEALLPREANYLAAIATGDGWGLAFLDVSTGEFKGTLLKSKSALYDELFRHRPAEVLLAPELRENEAFVAEFRKRFPVMLSEAPFEPQGEGPLALRRAQGALLAYARATQGGALSVRPFRLYDPGAFVRLPEASLKALEVFEPLRGQDTLFGVLDETRTAPGRRLLQAWLRHPLLERGPLEARLDRVERFVREGALREGVRRLLFRLADLERLATRLELSRASPRDLAALRRSLEILPELKGLLGEEVGLPDLSGLLEELRAALVEDPPLKVSEGGLIREGYDPDLDALRRAHAEGVAYFLDLEAREKERTGIPTLKVGYNAVFGYYLEVTRPYYEKVPQEYRPVQTLKDRQRYTLPEMKERERELYRLEALIKRREEEVFLALRERARKEAEALREAARILAELDVYAALAEVAVRHGYTRPRFGERLRIRAGRHPVVERRTAFVPNDLEMAHELVLVTGPNMAGKSTFLRQTALIALLAQIGSFVPAEEAELPLFDGIYTRIGASDDLAGGKSTFMVEMEEVALVLKEATERSLVLLDEVGRGTSSLDGVAIATALAEALHERRCYTLFATHYFELTALALPRLKNLHVAAKEEEGGLVFYHQVLPGPASKSYGVEVAEMAGLPKEVVERARALLSAMAARREGALEEVLERLLALDPDRLTPLEALRFLHELKALALGLPLGSMKG

SEQ ID NO: 4 - protein, 859 aa, Aquifex aeolicus
MEKSEKELTPMLSQYHYFKNQYPDCLLLFRLGDFYELFYEDAYIGSKELGLVLTSRPAGKGKERIPMCGVPYHSANSYIAKLVNKGYKVAICEQVEDPSKAKGIVKREVVRVITPGTFFERDTGGLASLYKKGNHYYVGYLNLAVGEFLGAKVKIEELLDLLSKLNIKEILVKKGEKLPEELEKVLKVYVSELEEEFFEEGSEEILKDFGVLSLQAFGFEEDTYSLPLGAVYKYAKTTQKGYTPLIPRPKPYRDEGFVRLDIKAIKGLEILESLEGRKDISLFKVIDRTLTGMGRRRLKFRLLSPFRSREKIERIQEGVQELKENREALLKIRQILEGMADLERLVSKISSNMATPRELVYLKNSLKKVEELRLLLLELKAPIFKEILQNFEDTKKIINDIEKTLVEDPPLHVKEGGLIREGVNAYLDELRFIRDNAETYLREYEKKLRQETGIQSLKIGYNKVMGYYIEVTKPNLKYVPSYFRRRQTLSNSERFTTEELQRLEEKILSAQTRINDLEYELYKELRERVVKELDKVGNNASAVAEVDFIQSLAQIAYEKDWAKPQIHEGYELIIEEGRHPVIEEFVENYVPNDTKLDRDSFIHVITGPNMAGKSSYIRQVGVLTLLSHIGSFIPARRAKIPVVDALFTRIGSGDVLALGVSTFMNEMLEVSNILNNATEKSLVILDEVGRGTSTYDGIAISKAIVKYISEKLKAKTLLATHFLEITELEGKIEGVKNYHMEVEKTPEGIRFLYILKEGKAEGSFGIEVAKLAGLPEEVVEEARKILRELEEKENKKEDIVPLLEETFKKSEEAQRLEEYEEIIKKIEEIDIGNTTPLQALLILAELKKKCSFSKKESGA

SEQ ID NO: 5 - protein, 855 aa, Aquifex pyrophilus
MGKEEKELTPMLAQYHQFKSMYPDCLLLFRLGDFYELFYEDAVVGSKELGLVLTSRPAGKGRERIPMCGVPYHSANNYIAKLVNKGYKVAICEQVEDPSKAKGIVKRDVIRVITPGTFFERETGGLCSLYRKGKSYLVSYLNLSVGEFIGAKVKEEELIDFLSKFNIREVLVKKGEKLPEKLEKVLKLHITELEEEFFEEGKEELLKDYGVPSIKAFGFQDEDLSLSLGAVYRYAKATQKSFTPLIPKPKPYVDEGYVKLDLKAVKGLEITESIEGRKDLSLFKVVDRTLTGMGRRRLRFRLLNPFRSIERIRKVQEAVEELINKREVLNEIRKTLEGMSDLERLVSRISSNMASPRELIHLKNSLRKAEELRKILSLLDSEIFKEIEGSLLNLNKVADLIDKTLVDDPPLHVKEGGLIKPGVNAYLDELRFIRENAEKLLKEYEKKLKKETGIQSLKIGYNKVMGYYIEVTKANVKYVPEHFRRRQTLSNAERYTTEELQRLEEKILSAQTRINELEYELYRELREEVVKELDKVGNNATLIGEVDYIQSLAWLALEKGWVKPEVHEGYELIIEEGKHPVIEEFTKNYVPNDTKLTEEEFIHVITGPNMAGKSSYIRQVGVLTLLAHTGSFLPVKSARIPLVDAIFTRIGSGDVLALGVSTFMNEMLDVSNILNNATKRSLIILDEVGRGTSTYDGIAISKAIVKYISEKIGAKTLLATHYLELTELERKVKGVKNYHMEVEETDEGIRFLYILKEGRAKGSFGIDVAKLAGLPEEVVREAKKILKELEGEKGKQEVLPFLEETYKKSVDEEKLNFYEEIIKEIEEIDIGNTTPVKALLILAELKERIKSFIKR

SEQ ID NO: 6 - protein, 793 aa, Thermotoga maritima
MKVTPLMEQYLRIKEQYKDSILLFRLGDFYEAFFEDAKIVSKVLNIVLTRRQDAPMAGIPYHALNTYLKKLVEAGYKVAICDQMEEPSKSKKLIRREVTRVVTPGSIVEDEFLSETNNYMAVVSEEKGRYCTVFCDVSTGEVLVHESSDEQETLDLLKNYSISQIICPEHLKSSLKERFPGVYTETISEWYFSDLEEVEKAYNLKDIHHFELSPLALKALAALIKYVKYTMIGEDLNLKPPLLISQRDYMILDSATVENLSWIPGDRGKNLFDVLNNTETPMGARLGKKWILHPLVDRKQIEERLKAVERLVNDRVSLEEMRNLLSNVRDVERIVSRVEYNRSVPRDLVALRETLEIIPKLNEVLSTFGVFKKLAFPEGLVDLLRKAIEDDPVGSPGEGKVIKRGFSSELDEYRDLLEHAEERLKEFEEKERERTGIQKLRVGYNQVFGYYIEVTKANLDKIPDDYERKQTLVNSERFITPELKEFETKIMAAKERIEELEKELFTSVCEEVKKHKEVLLEISEDLAKIDALSTLAYDAIMYNYTKPVFSEDRLEIKGGRHPVVERFTQNFVENDIYMDNEKRFVVITGPNMSGKSTFIRQVGLISLMAQIGSFVPAQKAILPVFDRIFTRMGARDDLAGGRSTFLVEMNEMALILLKSTNKSLVLLDEVGRGTSTQDGVSIAWAISEELIKRGCKVLFATHFTELTELEKHFPQVQNKTILVKEEGKNVIFTHKVVDGVADRSYGIEVAKIAGIPDRVINRAYEILERNFKNNTKKNGKSNRFSQQIPLFPV